European Patent Specification EP 3 342 865 B1, published September 20, 2023. Title: Ebola Virus Disease Vaccine Taking Human Replication Deficient Adenovirus As Vector. Applicant: Institute Of Biotechnology, Academy Of Military Medical Science,PLA. The sequence listing filed with the application follows.

SEQUENCE LISTING (2 sequences)

SEQ ID NO: 1 - DNA, 2037 bp, Ebola virus
atcgaattcgccgccaccatggacgccatgaagcggggcctctgctgtgttctgctgctctgcggcgccgtgttcgtgagtaactcgatccctctgggcgtcatccataattccaccctgcaagtgtccgacgtggacaagctcgtgtgccgcgacaagctgtccagtaccaatcagctccgatccgtcggtctcaacctggagggcaacggtgtcgccaccgatgtgccctccgccacgaagcggtggggcttcagatcgggcgtgcctccaaaggtcgtaaactacgaagccggcgaatgggccgagaactgttacaatctggagatcaaaaagcctgatggaagtgagtgtctccccgcagcccctgacggaatccgaggttttccaaggtgcagatatgtgcacaaggtctccggcaccgggccgtgcgcgggagacttcgcattccacaaagagggggcttttttcctgtacgaccggctggcgtccacggtaatttaccggggaacaaccttcgccgagggcgtggtcgccttcctcatcctgcctcaggctaagaaggatttcttctccagccaccccctgcgcgagcctgtgaacgccacagaggacccctctagtggctattatagtaccacaatccggtaccaggccaccggcttcggtaccaatgagaccgagtacctctttgaggtggataacctcacctacgtgcagctggagagtcgcttcaccccacagtttctgctgcagctgaatgagaccatctatgcctccgggaagcgctccaacaccacaggcaagctgatctggaaggtgaaccccgaaattgatacaacaatcggggagtgggctttctgggagaccaagaagaacctcaccagaaagatccgatccgaagagctgtccttcacagcggtctcgaatggccccaagaacatatccggccagtcacctgcccgcaccagttccgaccccgaaaccaacactaccaacgaggaccacaagatcatggcatccgagaacagttcggcaatggtacaggtgcacagtcagggtcgaaaggccgccgtgtcacacctcaccaccctcgccactatctccacttcgccccagagtctgaccaccaagccaggccccgataactccacgcataacacaccagtgtacaagctcgacatctccgaggccacgcaggtcgggcagcaccaccgccgggccgataacgatagcacggcatcggacacccctccagccaccaccgctgccgggcctctgaaggcagaaaataccaacacatctaaatccgcagactccctggacctggccaccactacctctccccaaaactattctgaaacagcaggcaacaataatacccaccaccaggacaccggggaggagtccgcctcttccggcaagctgggcctgattaccaacaccatcgccggcgtggccgggctgattacgggcggacggcggactcgacgggaggtcatcgtgaatgcccaacccaagtgtaacccgaacctccattattggaccacgcaggacgaaggcgctgctatcggcctcgcctggataccctactttggccccgccgccgagggtatctacactgagggcctcatgcacaatcaggatggcctgatctgtgggctcagacagctggccaacgagaccacccaggccctccagttattcttaagagccaccaccgagctgcggacgttctctatcctcaacagaaaagctattgacttcctgctccagcgatggggcggtacctgtcacatcctggggcccgactgctgcattgagccccacgactggacaaaaaacataaccgataagatcgatcagatcatccacgatttcgtggacaagaccctccccgaccagggcgataacgacaactggtggacaggctggcggcagtggatacccgccggtatcggggtgaccggtgtgatcattgccgtcatcgcgctgttctgcatctgcaagtttgtgttttagagatctaagcttgag

SEQ ID NO: 2 - DNA, 2064 bp, Ebola virus
atcgaattcgccgccaccatgggtgttacaggaatattgcagttacctcgtgatcgattcaagaggacatcattctttctttgggtaattatccttttccaaagaacattttccatcccgcttggagttatccacaatagtacattacaggttagtgatgtcgacaaactagtttgtcgtgacaaactgtcatccacaaatcaattgagatcagttggactgaatctcgaggggaatggagtggcaactgacgtgccatctgcgactaaaagatggggcttcaggtccggtgtcccaccaaaggtggtcaattatgaagctggtgaatgggctgaaaactgctacaatcttgaaatcaaaaaacctgacgggagtgagtgtctaccagcagcgccagacgggattcggggcttcccccggtgccggtatgtgcacaaagtatcaggaacgggaccatgtgccggagactttgccttccacaaagagggtgctttcttcctgtatgatcgacttgcttccacagttatctaccgaggaacgactttcgctgaaggtgtcgttgcatttctgatactgccccaagctaagaaggacttcttcagctcacaccccttgagagagccggtcaatgcaacggaggacccgtcgagtggctattattctaccacaattagatatcaggctaccggttttggaactaatgagacagagtacttgttcgaggttgacaatttgacctacgtccaacttgaatcaagattcacaccacagtttctgctccagctgaatgagacaatatatgcaagtgggaagaggagcaacaccacgggaaaactaatttggaaggtcaaccccgaaattgatacaacaatcggggagtgggccttctgggaaactaaaaaaaacctcactagaaaaattcgcagtgaagagttgtctttcacagctgtatcaaacggacccaaaaacatcagtggtcagagtccggcgcgaacttcttccgacccagagaccaacacaacaaatgaagaccacaaaatcatggcttcagaaaattcctctgcaatggttcaagtgcacagtcaaggaaggaaagctgcagtgtcgcatctgacaacccttgccacaatctccacgagtccccaatccctcacaaccaaaccaggtccggacaacagcacccataatacacccgtgtataaacttgacatctctgaggcaactcaagttggacaacatcaccgtagagcagacaacgacagcacagcctccgacactccccccgccacgaccgcagccggacccttaaaagcagagaacaccaacacgagtaagagcgctgactccctggacctcgccaccacgacaagcccccaaaactacagcgagactgctggcaacaacaacactcatcaccaagataccggagaagagagtgccagcagcgggaagctaggcttaattaccaatactattgctggagtagcaggactgatcacaggcgggagaaggactcgaagagaagtaattgtcaatgctcaacccaaatgcaaccccaatttacattactggactactcaggatgaaggtgctgcaatcggattggcctggataccatatttcgggccagcagccgaaggaatttacacagaggggctaatgcacaaccaagatggtttaatctgtgggttgaggcagctggccaacgaaacgactcaagctctccaactgttcctgagagccacaactgagctgcgaaccttttcaatcctcaaccgtaaggcaattgacttcctgctgcagcgatggggtggcacatgccacattttgggaccggactgctgtatcgaaccacatgattggaccaagaacataacagacaaaattgatcagattattcatgattttgttgataaaacccttccggaccagggggacaatgacaattggtggacaggatggagacaatggataccggcaggtattggagttacaggtgttataattgcagttatcgctttattctgtatatgcaaatttgtcttttagagatctaagcttgag